European Patent Application EP 4 134 444 A1, published February 15, 2023. Title: METHODS FOR TARGETED NUCLEIC ACID SEQUENCE ENRICHMENT WITH APPLICATIONS TO ERROR CORRECTED NUCLEIC ACID SEQUENCING. Applicant: UNIVERSITY OF WASHINGTON. Application EP, filed March 23, 2018. The sequence listing filed with the application follows.

SEQUENCE LISTING (50 sequences)

SEQ ID NO: 1-2 - skipped (2 entries)

SEQ ID NO: 3 - DNA, 8692 bp, Homo sapiens
  misc_feature 1..8692: note = TP53 - tumor protein p53
  source 1..8692: mol_type = genomic DNA
atacaagagatgaaatcctccagggtgtgggatggggtgagatttccttttaggtactaaggttcaccaagaggttgtcagacagggtttggctgggccagcagagacttgacaactccctctacctaaccagctgcccaactgtagaaactaccaacccaccgaccaacagggagagggaacaagcaccctcaagggggtcaagttctagaccccatgtaataaaaggtggtttcaaggccagatgtacattatttcattaaccctcacaatgcactctgtgaggtaggtgcaaatgccagcatttcacagatatgggccttgaagttagagaaaattcaacagtgagggacagcttccctggttagtacggtgaagtgggcccctacctagaatgtggctgattgtaaactaacccttaactgcaagaacatttcttacatctcccaaacatccctcacagtaaaaaccttaaaatctaagctggtatgtcctactccccatcctcctccccacaacaaaacaccagtgcaggccaacttgttcagtggagccccgggacaaagcaaatggaagtcctgggtgcttctgacgcacacctattgcaagcaagggttcaaagacccaaaacccaaaatggcaggggagggagagatgggggtgggaggctgtcagtggggaacaagaagtggagaatgtcagtctgagtcaggcccttctgtcttgaacatgagttttttatggcgggaggtagactgaccctttttggacttcaggtggctgtaggagacagaagcagggaggagagatgacatcacatgagtgagagggtctgtgccccttttccctgaccaatgctttgaagggcctaaggctgggacaacgggaattcaaatcaagatggtggccacaccccatgcaaatatgtttactgagcacctcagagtattagtgtgtattagtctcgtaatcttcccttaccccattttactttatttatcttttttgagacggagtttcactcttgttgcccaggctggagtgtaatggtgagatctcagctcaccgcaacctctgcctcccgggttcaagcgattctcctgcctcagcctcccgagtaggtagctgggattacaggcatgcatcaccacgcccggctacttttgtatttttagtagagatggggtttctccatgttggtcaggctgggctcaaactcccgacctcaggtgatccactcgccttggcctcccagagtgtgggattcgtgagccactgcgcccggcccccttaccccattttatatataaggaaactgagtttgacgggggtcacctaggacctgccggtgcatggcagggctgagtatatgacctgaaactctggctgtattcagtattacacaattattaggcccctccttgagaccctccagctctgggctgggagttgcggagaatggcaaagaagtatccacactcgtccctgggtttggatgttctgtggatacactgaggcaagaatgtggttataggattcaaccggaggaagactaaaaaaatgtctgtgcagggctgggacccaatgagatggggtcagctgcctttgaccatgaaggcaggatgagaatggaatcctatggctttccaacctaggaaggcaggggagtagggccaggaaggggctgaggtcactcacctggagtgagccctgctcccccctggctccttcccagcctgggcatccttgagttccaaggcctcattcagctctcggaacatctcgaagcgctcacgcccacggatctgcagcaacagaggagggggagaagtaagtatatacacagtacctgagttaaaagatggttcaagttacaattgtttgactttatgacggtacaaaagcaacatgcatttagtagaaactgcacttcaagtacctatacagctgacttttaaaaatatttatttatttattttgagatggggtctcactctgttgcccaggcgggagtgcaatggtgcaatcttggctgattgcaatctccgcctctggggttcaagtgattcttgtgcctcagcctcccgagtagctgggactacaggcgtgtgctaccacacctggctaatttttgtgtttttagtagagatggggcttcaccatgttagccaggctggtttccaactcctgacgtcaggtgatctacccacctccacctcccaaagtgctgggattacaggtgtgagccactgtgcccggcccttttttaaattttagagatgatgtcttgctatgttgttcaggctggactcaaactcttgggctcaagagatcctcctgccttagcctctcaagtaactgggactacatgtgcatgcgactgtgcctcgtttcttttcttttttttctgagacggagtctcactctatcgcccaggctggagtgcagtggcgccatcttggctccctgcaacctccgcctcctggttcaagcgattctcctgcctcagcctcccaagtagctgggattacaggcacctgccatcacgcccggttaatttttgtattttagtagagacggggtttcaccatgttggctaggctggtcttgaactcctgacctcaggtgatccacccgcctcagcctcccgaaatgctgggattacaggcgtgagccagtgcgcctggccttttctttttttgagtctcgctctgcgcccaggctgtgcctggctcgactgtgcctcctttcatgcaaccatgctgtttctcactttcagtaacaatattcaataaatcacatgagatatacaacattttattactataaaaagggctttgtgttagatgactttgcccaactgtagggtaacttaaatgctctgaacacgtttcaagtaggctagggctgagtgtggtagctcatgcctgtaaccccaatacttggggaggctgaggtggaaggattgattgagcccaggggtttgataccagcatgggcaacgtagcaagaccttgacttcacagaaaataaaaaattagctgggtgtcgtggcatgtgcctgtagtcctagctacttgggagggtgaaatcaccggagcccagggaggtcaaggctgcagtgagctgagatggtgccactgcactctagcctgagtgacagagtgagactctgtctttaaataaataaataaaaattagccgggcgtggtggctcacacctgtaatcccagcactttgggaggccgaggcgggcggatcacatggtcagaagttcgagaccagcctggccaacatggtgaaaccctgtctctactaaaaatacaaaaattagctgggcgtggtagcaggcgcttgtagtcctagctattcgggaggctgaggcaggagaatcacttgaacccaggaggcagaggttgcagtgagccgagatcatgccactgcactccagcctgggcgacagagtgagactgagtctcaaaaaaataaaataaaataaaataaaaataaataaataaaaattagccaggcatggtggtgcaggcctgtagttgaagcaacttgggaggctgagctgggaggatggatggagcctgggaggtggaggctgcagtgagctgtgactgcactactgcactctatccagcctgggtgacagagcaagaccttgtctcaaaaaagtaggctagagaccagcctgggcaacatagtgagactctatctatctacaaaaaattttaaaaattagctgggtatggtggtgtatgcctgtggtcctagctactggggaggcagagttagggggattgcttgagcccaggagggtataatgagctatgatcacatcactgtaatccagcctgggcaacagagcaagatgctgtctccattaaaaataaaataaaagtaggctaggcaggccgggtgcggtggctcacgcctgtaatcccagcactttgggaggccaaggcaggcagatcacaaggtcaggagttcgagactagcctggccaacatggtgaaacctcatctctactaaaaaaaaaaataaataaataacaaaaaattagctgggcgtcggggcaggtgcctgtaatcccagctactcagtgggctgaggcaggagaatcgcttgaacccagaaggcggaggttgcagtgagccgagatcccgccactgcactccagcctgggtgacagagtgagactctgtctccaaaaaaaaaaaaaaaaaaagcaggctaggctaagctatgatgttccttagattaggtgtattaaatccattttcaacttacaatattttcaacttacgacgagtttatcaggaagtaacaccatcgtaagtcaagtagcatctgtatcaggcaaagtcatagaaccattttcatgctctctttaacaattttctttttgaaagctggtctggtcctttaaaatatatattatggtataagttggtgttctgaagttagttagctacaaccaggagccattgtctttgaggcatcactgccccctgatggcaaatgccccaattgcaggtaaaacagtcaagaagaaaacggcattttgagtgttagactggaaactttccacttgataagaggtcccaagacttagtacctgaagggtgaaatattctccatccagtggtttcttctttggctggggagaggagctggtgttgttgggcagtgctaggaaagaggcaaggaaaggtgataaaagtgaatctgaggcataactgcacccttggtctcctccaccgcttcttgtcctgcttgcttacctcgcttagtgctccctgggggcagctcgtggtgaggctcccctttcttgcggagattctcttcctctgtgcgccggtctctcccaggacaggcacaaacacgcacctcaaagctgttccgtcccagtagattaccactactcaggataggaaaagagaagcaagaggcagtaaggaaatcaggtcctacctgtcccatttaaaaaaccaggctccatctactcccaaccacccttgtcctttctggagcctaagctccagctccaggtaggtggaggagaagccacaggttaagaggtcccaaagccagagaaaagaaaactgagtgggagcagtaaggagattccccgccggggatgtgatgagaggtggatgggtagtagtatggaagaaatcggtaagaggtgggcccaggggtcagaggcaagcagaggctggggcacagcaggccagtgtgcagggtggcaagtggctcctgacctggagtcttccagtgtgatgatggtgaggatgggcctccggttcatgccgcccatgcaggaactgttacacatgtagttgtagtggatggtggtacagtcagagccaacctaggagataacacaggcccaagatgaggccagtgcgccttggggagacctgtggcaagcaggggaggccttttttttttttttttgagatggaatctcgctctgtcgcccaggctggagtgcagtggcgtgatctcagctcactgcaagctccaccgcccaggttcacgccattctccttcctcagcctcccgagtagctgggactacaggtgcccagcaccacgcccggctaatttttttttgtatttttcagtagagacggggtttcaccgttagccaggatggtctcgatctcccaacctcgtgatccgcctgccttggcctcccaaagtgctgggattacaggcatgagccactgcgcccagccaagcaggggaggcccttagcctctgtaagcttcagttttttcaactgtgcaatagttaaacccatttactttgcacatctcatggggttatagggaggtcaaataagcagcaggagaaagcccccctactgctcacctggagggccactgacaaccacccttaacccctcctcccagagaccccagttgcaaaccagacctcaggcggctcatagggcaccaccacactatgtcgaaaagtgtttctgtcatccaaatactccacacgcaaatttccttccactcggataagatgctgaggaggggccagacctaagagcaatcagtgaggaatcagaggcctggggaccctgggcaaccagccctgtcgtctctccagccccagctgctcaccatcgctatctgagcagcgctcatggtgggggcagcgcctcacaacctccgtcatgtgctgtgactgcttgtagatggccatggcgcggacgcgggtgccgggcgggggtgtggaatcaacccacagctgcacagggcaggtcttggccagttggcaaaacatcttgttgagggcaggggagtactgtaggaagaggaaggagacagagttgaaagtcagggcacaagtgaacagataaagcaactggaagacggcagcaaagaaacaaacatgcgtaagcacctcctgcaacccactagcgagctagagagagttggcgtctacacctcaggagcttttcttttttttttttttttttgagatagggtcttgctctgtcactcaggctggagcacagtggtgtgatcacagctcactgcagcctccatctcctggcctcaagtgatcttcccacctcagcctcctaagtggctgggactataggtgtgcaccaccatgcctggctaattttttgtatttttttgtagagacgaggtttcatcatgttacccaggctggtcttgaactcctgggctcaggtgatctgcctgccttggcctctttgagagtgctgggattgcaggtgtgagccaccaagcctggtcaggagcttattttcaaaagccaaggaatacacgtggatgaagaaaaagaaaagttctgcatccccaggagagatgctgagggtgtgatgggatggataaaagcccaaattcaaggggggaatattcaactttgggacaggagtcagagatcacacattaagtgggtaaactataaaaaaacactgacaggaagccaaagggtgaagaggaatcccaaagttccaaacaaaagaaatgcagggggatacggccaggcattgaagtctcatggaagccagcccctcagggcaactgaccgtgcaagtcacagacttggctgtcccagaatgcaagaagcccagacggaaaccgtagctgccctggtaggttttctgggaagggacagaagatgacaggggccaggagggggctggtgcaggggccgccggtgtaggagctgctggtgcaggggccacggggggagcagcctctggcattctgggagcttcatctggacctgggtcttcagtgaaccattgttcaatatcgtccggggacagcatcaaatcatccattgcttgggacggcaagggggactgtagatgggtgaaaagagcagtcagaggaccaggtcctcagccccccagccccccagccctccaggtccccagccctccaggtccccagcccaacccttgtccttaccagaacgttgttttcaggaagtctgaaagacaagagcagaaagtcagtcccatggaattttcgcttcccacaggtctctgctagggggctggggttggggtgggggtggtgggcctgcccttccaatggatccactcacagtttccataggtctgaaaatgtttcctgactcagagggggctcgacgctaggatctgactgcggctcctccatggcagtgacccggaaggcagtctggctgctgcaagaggaaaagtggggatccagcatgagacacttccaaccctgggtcacctgggcctgcagagaaggaaccccctcccccaacaccatgccagtgtctgagacagctcggcttcctgtggagcaggaaaagaatggctgcttcacattctctcttccaatgtttcaccacaacccaagcactcctgccccacccctcaccagccatgcacttctttgaggaaaagacaatcagagagggacttccaaccttcccaccactaaatccccaagacttcctaaatgtgcaccctattcccaactcccttcctgtattttttttttttttttgagatggagtctctctctgtcacctaggctggagcacagtggcatgatctcagctcactgcaacctctaccttccgggttcaagccattctcctgcctcagtctcccgagtagctgggattacaggcgagtaccaccacacccagctaatttttgtatttttagtagagacagggctttgcatgttggccaggctggtctcgaactccttacttcaggtgatcggcccgcctcagcctcctaaagtgccaagattacaggtgtgagctaccgtgccctgctcccacctcctgttaacaaggatatagtcattctcagcctgcaatctctgtatggggaaggacacccccttggcccccacccttccccacctgatacacggctccatttctttgattcctttcactgcaaagcttctggaagaacaactgtctcaccgctcacctgcccattctcttcggacactcctcagccctgcattacaaacccctcacgaatggcccgtctcggcttctttaatctcatctcttaacaaccactccctcttccccaaaagctctagctagactggctgcccttctctgctaatcaactggtggttccttggctagccaggaacatgggggtaggctccttcccgtgcagactt

SEQ ID NO: 4 - DNA, 23 bp, synthetic construct
  misc_feature 1..23: note = Synthetic
  source 1..23: mol_type = other DNA
gtgggcccctacctagaatgtgg

SEQ ID NO: 5 - DNA, 23 bp, synthetic construct
  misc_feature 1..23: note = Synthetic
  source 1..23: mol_type = other DNA
attcccgttgtcccagccttagg

SEQ ID NO: 6 - DNA, 23 bp, synthetic construct
  misc_feature 1..23: note = Synthetic
  source 1..23: mol_type = other DNA
tggttataggattcaaccggagg

SEQ ID NO: 7 - DNA, 23 bp, synthetic construct
  misc_feature 1..23: note = Synthetic
  source 1..23: mol_type = other DNA
ctgattgcaatctccgcctctgg

SEQ ID NO: 8 - DNA, 23 bp, synthetic construct
  misc_feature 1..23: note = Synthetic
  source 1..23: mol_type = other DNA
cggcattttgagtgttagactgg

SEQ ID NO: 9 - DNA, 23 bp, synthetic construct
  misc_feature 1..23: note = Synthetic
  source 1..23: mol_type = other DNA
ctttgggacctcttaacctgtgg

SEQ ID NO: 10 - DNA, 23 bp, synthetic construct
  misc_feature 1..23: note = Synthetic
  source 1..23: mol_type = other DNA
caggtctccccaaggcgcactgg

SEQ ID NO: 11 - DNA, 23 bp, synthetic construct
  misc_feature 1..23: note = Synthetic
  source 1..23: mol_type = other DNA
gcacatctcatggggttataggg

SEQ ID NO: 12 - DNA, 23 bp, synthetic construct
  misc_feature 1..23: note = Synthetic
  source 1..23: mol_type = other DNA
caggggagtactgtaggaagagg

SEQ ID NO: 13 - DNA, 23 bp, synthetic construct
  misc_feature 1..23: note = Synthetic
  source 1..23: mol_type = other DNA
tgcacggtcagttgccctgaggg

SEQ ID NO: 14 - DNA, 23 bp, synthetic construct
  misc_feature 1..23: note = Synthetic
  source 1..23: mol_type = other DNA
atggaattttcgcttcccacagg

SEQ ID NO: 15 - DNA, 23 bp, synthetic construct
  misc_feature 1..23: note = Synthetic
  source 1..23: mol_type = other DNA
tgggaatagggtgcacatttagg

SEQ ID NO: 16 - DNA, 120 bp, synthetic construct
  misc_feature 1..120: note = Synthetic
  source 1..120: mol_type = other DNA
ccccgggacaaagcaaatggaagtcctgggtgcttctgacgcacacctattgcaagcaagggttcaaagacccaaaacccaaaatggcaggggagggagagatgggggtgggaggctgtc

SEQ ID NO: 17 - DNA, 120 bp, synthetic construct
  misc_feature 1..120: note = Synthetic
  source 1..120: mol_type = other DNA
agtggggaacaagaagtggagaatgtcagtctgagtcaggcccttctgtcttgaacatgagttttttatggcgggaggtagactgaccctttttggacttcaggtggctgtaggagacag

SEQ ID NO: 18 - DNA, 120 bp, synthetic construct
  misc_feature 1..120: note = Synthetic
  source 1..120: mol_type = other DNA
actcacctggagtgagccctgctcccccctggctccttcccagcctgggcatccttgagttccaaggcctcattcagctctcggaacatctcgaagcgctcacgcccacggatctgcagc

SEQ ID NO: 19 - DNA, 120 bp, synthetic construct
  misc_feature 1..120: note = Synthetic
  source 1..120: mol_type = other DNA
aatcctatggctttccaacctaggaaggcaggggagtagggccaggaaggggctgaggtcactcacctggagtgagccctgctcccccctggctccttcccagcctgggcatccttgagt

SEQ ID NO: 20 - DNA, 120 bp, synthetic construct
  misc_feature 1..120: note = Synthetic
  source 1..120: mol_type = other DNA
tccaaggcctcattcagctctcggaacatctcgaagcgctcacgcccacggatctgcagcaacagaggagggggagaagtaagtatatacacagtacctgagttaaaagatggttcaagt

SEQ ID NO: 21 - DNA, 120 bp, synthetic construct
  misc_feature 1..120: note = Synthetic
  source 1..120: mol_type = other DNA
aagaggtcccaagacttagtacctgaagggtgaaatattctccatccagtggtttcttctttggctggggagaggagctggtgttgttgggcagtgctaggaaagaggcaaggaaaggtg

SEQ ID NO: 22 - DNA, 120 bp, synthetic construct
  misc_feature 1..120: note = Synthetic
  source 1..120: mol_type = other DNA
gcataactgcacccttggtctcctccaccgcttcttgtcctgcttgcttacctcgcttagtgctccctgggggcagctcgtggtgaggctcccctttcttgcggagattctcttcctctg

SEQ ID NO: 23 - DNA, 120 bp, synthetic construct
  misc_feature 1..120: note = Synthetic
  source 1..120: mol_type = other DNA
tgcgccggtctctcccaggacaggcacaaacacgcacctcaaagctgttccgtcccagtagattaccactactcaggataggaaaagagaagcaagaggcagtaaggaaatcaggtccta

SEQ ID NO: 24 - DNA, 120 bp, synthetic construct
  misc_feature 1..120: note = Synthetic
  source 1..120: mol_type = other DNA
tgacctggagtcttccagtgtgatgatggtgaggatgggcctccggttcatgccgcccatgcaggaactgttacacatgtagttgtagtggatggtggtacagtcagagccaacctagga

SEQ ID NO: 25 - DNA, 120 bp, synthetic construct
  misc_feature 1..120: note = Synthetic
  source 1..120: mol_type = other DNA
atgtgatgagaggtggatgggtagtagtatggaagaaatcggtaagaggtgggcccaggggtcagaggcaagcagaggctggggcacagcaggccagtgtgcagggtggcaagtggctcc

SEQ ID NO: 26 - DNA, 120 bp, synthetic construct
  misc_feature 1..120: note = Synthetic
  source 1..120: mol_type = other DNA
gacctcaggcggctcatagggcaccaccacactatgtcgaaaagtgtttctgtcatccaaatactccacacgcaaatttccttccactcggataagatgctgaggaggggccagacctaa

SEQ ID NO: 27 - DNA, 120 bp, synthetic construct
  misc_feature 1..120: note = Synthetic
  source 1..120: mol_type = other DNA
ctggagggccactgacaaccacccttaacccctcctcccagagaccccagttgcaaaccagacctcaggcggctcatagggcaccaccacactatgtcgaaaagtgtttctgtcatccaa

SEQ ID NO: 28 - DNA, 120 bp, synthetic construct
  misc_feature 1..120: note = Synthetic
  source 1..120: mol_type = other DNA
caccatcgctatctgagcagcgctcatggtgggggcagcgcctcacaacctccgtcatgtgctgtgactgcttgtagatggccatggcgcggacgcgggtgccgggcgggggtgtggaat

SEQ ID NO: 29 - DNA, 120 bp, synthetic construct
  misc_feature 1..120: note = Synthetic
  source 1..120: mol_type = other DNA
gaatcagaggcctggggaccctgggcaaccagccctgtcgtctctccagccccagctgctcaccatcgctatctgagcagcgctcatggtgggggcagcgcctcacaacctccgtcatgt

SEQ ID NO: 30 - DNA, 120 bp, synthetic construct
  misc_feature 1..120: note = Synthetic
  source 1..120: mol_type = other DNA
caacccacagctgcacagggcaggtcttggccagttggcaaaacatcttgttgagggcaggggagtactgtaggaagaggaaggagacagagttgaaagtcagggcacaagtgaacagat

SEQ ID NO: 31 - DNA, 120 bp, synthetic construct
  misc_feature 1..120: note = Synthetic
  source 1..120: mol_type = other DNA
attgaagtctcatggaagccagcccctcagggcaactgaccgtgcaagtcacagacttggctgtcccagaatgcaagaagcccagacggaaaccgtagctgccctggtaggttttctggg

SEQ ID NO: 32 - DNA, 120 bp, synthetic construct
  misc_feature 1..120: note = Synthetic
  source 1..120: mol_type = other DNA
aagggacagaagatgacaggggccaggagggggctggtgcaggggccgccggtgtaggagctgctggtgcaggggccacggggggagcagcctctggcattctgggagcttcatctggac

SEQ ID NO: 33 - DNA, 120 bp, synthetic construct
  misc_feature 1..120: note = Synthetic
  source 1..120: mol_type = other DNA
ctgggtcttcagtgaaccattgttcaatatcgtccggggacagcatcaaatcatccattgcttgggacggcaagggggactgtagatgggtgaaaagagcagtcagaggaccaggtcctc

SEQ ID NO: 34 - DNA, 120 bp, synthetic construct
  misc_feature 1..120: note = Synthetic
  source 1..120: mol_type = other DNA
gccccccagccctccaggtccccagccctccaggtccccagcccaacccttgtccttaccagaacgttgttttcaggaagtctgaaagacaagagcagaaagtcagtcccatggaatttt

SEQ ID NO: 35 - DNA, 120 bp, synthetic construct
  misc_feature 1..120: note = Synthetic
  source 1..120: mol_type = other DNA
cgcttcccacaggtctctgctagggggctggggttggggtgggggtggtgggcctgcccttccaatggatccactcacagtttccataggtctgaaaatgtttcctgactcagagggggc

SEQ ID NO: 36 - DNA, 120 bp, synthetic construct
  misc_feature 1..120: note = Synthetic
  source 1..120: mol_type = other DNA
tcgacgctaggatctgactgcggctcctccatggcagtgacccggaaggcagtctggctgctgcaagaggaaaagtggggatccagcatgagacacttccaaccctgggtcacctgggcc

SEQ ID NO: 37 - DNA, 500 bp, synthetic construct
  misc_feature 1..500: note = Synthetic
  source 1..500: mol_type = other DNA
gctgagtgtgggcccctacctagaatgtgggacggagtctcactctaattcccgttgtcccagccttaggcccaggctggagtgcagtggttataggattcaaccggaggcgccatcttggctccctctgattgcaatctccgcctctggacctccgcctcctggttcggcattttgagtgttagactgggattctcctgcctcagcctttgggacctcttaacctgtggccaagtagctgggattacaggtctccccaaggcgcactgggcacctgccatcacgccgcacatctcatggggttataggggtagagacggggtttcacaggggagtactgtaggaagaggtgttggctaggctggtctgcacggtcagttgccctgagggaactcctgacctcaggtatggaattttcgcttcccacaggtcagcctcccgaaatgctgggaatagggtgcacatttagggtggtagctcatgcctgtaaccccaatgtc

SEQ ID NO: 38 - DNA, 17 bp, synthetic construct
  misc_feature 1..17: note = Synthetic
  source 1..17: mol_type = other DNA
gacggagtctcactcta

SEQ ID NO: 39 - DNA, 17 bp, synthetic construct
  misc_feature 1..17: note = Synthetic
  source 1..17: mol_type = other DNA
cccaggctggagtgcag

SEQ ID NO: 40 - DNA, 17 bp, synthetic construct
  misc_feature 1..17: note = Synthetic
  source 1..17: mol_type = other DNA
cgccatcttggctccct

SEQ ID NO: 41 - DNA, 17 bp, synthetic construct
  misc_feature 1..17: note = Synthetic
  source 1..17: mol_type = other DNA
acctccgcctcctggtt

SEQ ID NO: 42 - DNA, 17 bp, synthetic construct
  misc_feature 1..17: note = Synthetic
  source 1..17: mol_type = other DNA
gattctcctgcctcagc

SEQ ID NO: 43 - DNA, 17 bp, synthetic construct
  misc_feature 1..17: note = Synthetic
  source 1..17: mol_type = other DNA
ccaagtagctgggatta

SEQ ID NO: 44 - DNA, 17 bp, synthetic construct
  misc_feature 1..17: note = Synthetic
  source 1..17: mol_type = other DNA
gcacctgccatcacgcc

SEQ ID NO: 45 - DNA, 17 bp, synthetic construct
  misc_feature 1..17: note = Synthetic
  source 1..17: mol_type = other DNA
gtagagacggggtttca

SEQ ID NO: 46 - DNA, 17 bp, synthetic construct
  misc_feature 1..17: note = Synthetic
  source 1..17: mol_type = other DNA
tgttggctaggctggtc

SEQ ID NO: 47 - DNA, 17 bp, synthetic construct
  misc_feature 1..17: note = Synthetic
  source 1..17: mol_type = other DNA
aactcctgacctcaggt

SEQ ID NO: 48 - DNA, 17 bp, synthetic construct
  misc_feature 1..17: note = Synthetic
  source 1..17: mol_type = other DNA
tcagcctcccgaaatgc

SEQ ID NO: 49 - skipped

SEQ ID NO: 50 - DNA, 30 bp, synthetic construct
  misc_feature 1..30: note = Synthetic
  source 1..30: mol_type = other DNA
gtggtagctcatgcctgtaaccccaatgtc